European Patent Specification EP 4 294 454 B1, published April 15, 2026. Title: ANTI-VIRAL PEPTIDES AND COMPOSITIONS AND METHODS OF USE THEREOF. Applicant: Versitech Limited Centre for Virology, Vaccinology and Therapeutics Limited. The sequence listing filed with the application follows.

SEQUENCE LISTING (11 sequences)

SEQ ID NO: 1 - protein, 16 aa, Artificial Sequence
  Amino acid sequence of P16 peptide
RGAHIKGRWKSRCHRF

SEQ ID NO: 2 - protein, 27 aa, Rana nigromaculata
IPLRGAFINGRWDSQCHRFSNGAIACA

SEQ ID NO: 3 - protein, 21 aa, Rana nigromaculata
FINGRWDSQCHRFSNGAIACA

SEQ ID NO: 4 - protein, 20 aa, Rana nigromaculata
IPLRGAFINGRWDSQCHRFS

SEQ ID NO: 5 - protein, 13 aa, Rana nigromaculata
IPLRGAFINGRWD

SEQ ID NO: 6 - protein, 14 aa, Rana nigromaculata
FINGRWDSQCHRFS

SEQ ID NO: 7 - protein, 16 aa, Rana nigromaculata
WDSQCHRFSNGAIACA

SEQ ID NO: 8 - DNA, 30 bp, Artificial Sequence
  Primer
cctactaaattaaatgatctctgctttact

SEQ ID NO: 9 - DNA, 21 bp, Artificial Sequence
  Primer
caagctataacgcagcctgta

SEQ ID NO: 10 - DNA, 21 bp, Artificial Sequence
  Primer
cttctaaccgaggtcgaaacg

SEQ ID NO: 11 - DNA, 22 bp, Artificial Sequence
  Primer
ggcattttggacaaakcgtcta